European Patent Application EP 4 273 249 A2, published November 8, 2023. Title: IMPROVED EXPRESSION OF RECOMBINANT PROTEINS. Applicant: NOVOZYMES A/S. The sequence listing filed with the application follows.

SEQUENCE LISTING (188 sequences)

SEQ ID NO: 1 - DNA, 84 bp, Bacillus pumilus
  source 1..84: mol_type = genomic DNA
atgaaatttaaaacgttatcagtagtattcgtgatgattagtgtcataagtgttgttagttattttacgtcagaagtgacagcg

SEQ ID NO: 2 - DNA, 80 bp, Bacillus pumilus
  source 1..80: mol_type = genomic DNA
atgatgaaaaaagtaagtggcttaatcatattatcgatgatgctgttgtctggtttttatatggaaacagcttatggtgc

SEQ ID NO: 3 - protein, 28 aa, Bacillus pumilus
MKFKTLSVVFVMISVISVVSYFTSEVTA

SEQ ID NO: 4 - protein, 27 aa, Bacillus pumilus
MMKKVSGLIILSMMLLSGFYMETAYGA

SEQ ID NO: 5 - DNA, 21 bp, Nocardiopsis prasina
  source 1..21: mol_type = other DNA
acaggagcattaccgcagtct

SEQ ID NO: 6 - DNA, 21 bp, Bacillus clausii
  source 1..21: mol_type = other DNA
gctgaagaagcaaaagaaaaa

SEQ ID NO: 7 - protein, 7 aa, Nocardiopsis prasina
TGALPQS

SEQ ID NO: 8 - protein, 7 aa, Bacillus clausii
AEEAKEK

SEQ ID NO: 9 - DNA, 105 bp, synthetic construct
  misc_feature 1..105: note = artificial sequence
  source 1..105: mol_type = other DNA
  sig_peptide 1..84
  misc_structure 85..105: note = SP-linker
atgaaatttaaaacgttatcagtagtattcgtgatgattagtgtcataagtgttgttagttattttacgtcagaagtgacagcgacaggagcattaccgcagtct

SEQ ID NO: 10 - DNA, 102 bp, synthetic construct
  source 1..102: mol_type = other DNA
  sig_peptide 1..81
  misc_feature 82..102: note = SP-linker
atgatgaaaaaagtaagtggcttaatcatattatcgatgatgctgttgtctggtttttatatggaaacagcttatggtgcggctgaagaagcaaaagaaaaa

SEQ ID NO: 11 - protein, 35 aa, synthetic construct
  SIGNAL 1..28
  REGION 29..35: note = SP-linker
MKFKTLSVVFVMISVISVVSYFTSEVTATGALPQS

SEQ ID NO: 12 - protein, 34 aa, synthetic construct
  SIGNAL 1..17
  REGION 18..34: note = SP-linker
MMKKVSGLIILSMMLLSGFYMETAYGAAEEAKEK

SEQ ID NO: 13 - DNA, 1539 bp, synthetic construct
  misc_feature 1..1539: note = amylase coding sequence
  source 1..1539: mol_type = other DNA
atgaaacaacaaaaacggctttacgcccgattgctgacgctgttatttgcgctcatcttcttgctgcctcattctgcagcagcggcggcaaatcttaatgggacgctgatgcagtattttgaatggtacatgcccaatgacggccaacattggaggcgtttgcaaaacgactcggcatatttggctgaacacggtattactgccgtctggattcccccggcatataagggaacgagccaagcggatgtgggctacggtgcttacgacctttatgatttaggggagtttcatcaaaaagggacggttcggacaaagtacggcacaaaaggagagctgcaatctgcgatcaaaagtcttcattcccgcgacattaacgtttacggggatgtggtcatcaaccacaaaggcggcgctgatgcgaccgaagatgtaaccgcggttgaagtcgatcccgctgaccgcaaccgcgtaatttcaggagaacacctaattaaagcctggacacattttcattttccggggcgcggcagcacatacagcgattttaaatggcattggtaccattttgacggaaccgattgggacgagtcccgaaagctgaaccgcatctataagtttcaaggaaaggcttgggattgggaagtttccaatgaaaacggcaactatgattatttgatgtatgccgacatcgattatgaccatcctgatgtcgcagcagaaattaagagatggggcacttggtatgccaatgaactgcaattggacggtttccgtcttgatgctgtcaaacacattaaattttcttttttgcgggattgggttaatcatgtcagggaaaaaacggggaaggaaatgtttacggtagctgaatattggcagaatgacttgggcgcgctggaaaactatttgaacaaaacaaattttaatcattcagtgtttgacgtgccgcttcattatcagttccatgctgcatcgacacagggaggcggctatgatatgaggaaattgctgaacggtacggtcgtttccaagcatccgttgaaatcggttacatttgtcgataaccatgatacacagccggggcaatcgcttgagtcgactgtccaaacatggtttaagccgcttgcttacgcttttattctcacaagggaatctggataccctcaggttttctacggggatatgtacgggacgaaaggagactcccagcgcgaaattcctgccttgaaacacaaaattgaaccgatcttaaaagcgagaaaacagtatgcgtacggagcacagcatgattatttcgaccaccatgacattgtcggctggacaagggaaggcgacagctcggttgcaaattcaggtttggcggcattaataacagacggacccggtggggcaaagcgaatgtatgtcggccggcaaaacgccggtgagacatggcatgacattaccggaaaccgttcggagccggttgtcatcaattcggaaggctggggagagtttcacgtaaacggcgggtcggtttcaatttatgttcaaagatag

SEQ ID NO: 14 - protein, 519 aa, synthetic construct
  REGION 1..7: note = SP-linker
TGALPQSMKQQKRLYARLLTLLFALIFLLPHSAAAAANLNGTLMQYFEWYMPNDGQHWRRLQNDSAYLAEHGITAVWIPPAYKGTSQADVGYGAYDLYDLGEFHQKGTVRTKYGTKGELQSAIKSLHSRDINVYGDVVINHKGGADATEDVTAVEVDPADRNRVISGEHLIKAWTHFHFPGRGSTYSDFKWHWYHFDGTDWDESRKLNRIYKFQGKAWDWEVSNENGNYDYLMYADIDYDHPDVAAEIKRWGTWYANELQLDGFRLDAVKHIKFSFLRDWVNHVREKTGKEMFTVAEYWQNDLGALENYLNKTNFNHSVFDVPLHYQFHAASTQGGGYDMRKLLNGTVVSKHPLKSVTFVDNHDTQPGQSLESTVQTWFKPLAYAFILTRESGYPQVFYGDMYGTKGDSQREIPALKHKIEPILKARKQYAYGAQHDYFDHHDIVGWTREGDSSVANSGLAALITDGPGGAKRMYVGRQNAGETWHDITGNRSEPVVINSEGWGEFHVNGGSVSIYVQR

SEQ ID NO: 15 - protein, 519 aa, synthetic construct
  REGION 1..7: note = SP-linker
AEEAKEKMKQQKRLYARLLTLLFALIFLLPHSAAAAANLNGTLMQYFEWYMPNDGQHWRRLQNDSAYLAEHGITAVWIPPAYKGTSQADVGYGAYDLYDLGEFHQKGTVRTKYGTKGELQSAIKSLHSRDINVYGDVVINHKGGADATEDVTAVEVDPADRNRVISGEHLIKAWTHFHFPGRGSTYSDFKWHWYHFDGTDWDESRKLNRIYKFQGKAWDWEVSNENGNYDYLMYADIDYDHPDVAAEIKRWGTWYANELQLDGFRLDAVKHIKFSFLRDWVNHVREKTGKEMFTVAEYWQNDLGALENYLNKTNFNHSVFDVPLHYQFHAASTQGGGYDMRKLLNGTVVSKHPLKSVTFVDNHDTQPGQSLESTVQTWFKPLAYAFILTRESGYPQVFYGDMYGTKGDSQREIPALKHKIEPILKARKQYAYGAQHDYFDHHDIVGWTREGDSSVANSGLAALITDGPGGAKRMYVGRQNAGETWHDITGNRSEPVVINSEGWGEFHVNGGSVSIYVQR

SEQ ID NO: 16 - protein, 353 aa, synthetic construct
  REGION 1..353: note = artificial sequence
AEEAKEKYLIGFNEQEAVSEFVEQVEANDEVAILSEEEEVEIELLHEFETIPVLSVELSPEDVDALELDPAISYIEEDAEVTTMAQSVPWGISRVQAPAAHNRGLTGSGVKVAVLDTGISTHPDLNIRGGASFVPGEPSTQDGNGHGTHVAGTIAALNNSIGVLGVAPSAELYAVKVLGASGSGSVSSIAQGLEWAGNNGMHVANLSLGSPSPSATLEQAVNSATSRGVLVVAASGNSGAGSISYPARYANAMAVGATDQNNNRASFSQYGAGLDIVAPGVNVQSTYPGSTYASLNGTSMATPHVAGAAALVKQKNPSWSNVQIRNHLKNTATSLGSTNLYGSGLVNAEAATR

SEQ ID NO: 17 - protein, 352 aa, synthetic construct
  REGION 1..352: note = artificial sequence
TGALPQSPTPEADAVSMQEALQRDLDLTSAEAEELLAAQDTAFEVDEAAAEAAGDAYGGSVFDTESLELTVLVTDAAAVEAVEATGAGTELVSYGIDGLDEIVQELNAADAVPGVVGWYPDVAGDTVVLEVLEGSGADVSGLLADAGVDASAVEVTTSDQPELYADIIGGLAYTMGGRCSVGFAATNAAGQPGFVTAGHCGRVGTQVTIGNGRGVFEQSVFPGNDAAFVRGTSNFTLTNLVSRYNTGGYATVAGHNQAPIGSSVCRSGSTTGWHCGTIQARGQSVSYPEGTVTNMTRTTVCAEPGDSGGSYISGTQAQGVTSGGSGNCRTGGTTFYQEVTPMVNSWGVRLRT

SEQ ID NO: 18 - protein, 45 aa, Bacillus pumilus
MKFKTLSVVFVMISVISVVSYFTSEVTASHDEARRGHTASIGYTA

SEQ ID NO: 19 - protein, 110 aa, Bacillus pumilus
MMKKVSGLIILSMMLLSGFYMETAYGETPQMEKRPVMHQVKLTTEQQKQIEMLEQQILSKRKEVIEKYVQYGVLTKEQGTHITKRMDEHYNHLENNGFVPLLKKPQHHRP

SEQ ID NO: 20 - DNA, 309 bp, synthetic construct
  misc_feature 1..309: note = artificial sequence
  source 1..309: mol_type = other DNA
ataaatgagtagaaagcgccatatcggcgcttttcttttggaagaaaatatagggaaaatggtacttgttaaaaattcggaatatttatacaatatcatatgtatcacattgaaaggaggggcctgctgtccagactgtccgctgtgtaaaaaaaaggaataaaggggggttgacattattttactgatatgtataatataatttgtataagaaaatggaggggccctcgaaacgtaagatgaaaccttagataaaagtgctttttttgttgcaattgaagaattattaatgttaagcttaattaaaga

SEQ ID NO: 21 - protein, 275 aa, Bacillus licheniformis
MYNVIGVRFKKAGKIYYFDPNGFQIDKDSCVIVETVRGVEYGQVVIANKKVDENDVVLPLRKVIRVADERDRLIVEENQEAALSAFDVCQKKVNEHGLEMKLVDVEFTFDRNKVIFYFTADGRVDFRELVKDLASIFKTRIELRQIGVRDEAKMLGGIGPCGRMLCCSTFLGDFEPVSIKMAKDQNLSLNPTKISGLCGRLMCCLKYENDEYETAKEQLPDIGEVIATSSGPAKVVGLNILERILQVELTDCDKVVEYTWDELLQEGVVSAQTTD

SEQ ID NO: 22 - protein, 172 aa, Bacillus licheniformis
MKKRFLVIAGVLLVIVVGIQVKNAVFIEYKVEGVSMNPTFQEGNELLINRFAHRFKTISRFDIVLFKGPDKDIFIKRVIGLPGETLRYEDDQLYINEEKIKEPYLDDLKAVTAGGDLTGDFTLQEVTGEEKVPENEYFVLGDNRIHSFDSRHFGFVSERDIVGIVTERIDKK

SEQ ID NO: 23 - protein, 186 aa, Bacillus licheniformis
MTEEKSTNKKNSLFEWVKAIIIAVVLALLIRAFLFEPYLVEGTSMDPTLHDGERLFVYKTVRYVGEFKRGDIVIIDGDEKNVHYVKRLIGLPGDTVQMKDDTLYINGKKVSEPYLSENRKEAEAVGVKLTGDFGPVKVPEGKYFVMGDNRQRSMDSRNGLGLIDKKRVAGTSQFVFFPFNEIRKTD

SEQ ID NO: 24 - protein, 4 aa, NOCARDIOPSIS PRASINA
TGAL

SEQ ID NO: 25 - protein, 5 aa, NOCARDIOPSIS PRASINA
TGALP

SEQ ID NO: 26 - protein, 6 aa, NOCARDIOPSIS PRASINA
TGALPQ

SEQ ID NO: 27 - protein, 7 aa, Nocardiopsis prasina
TGALPQS

SEQ ID NO: 28 - protein, 8 aa, Nocardiopsis prasina
TGALPQSP

SEQ ID NO: 29 - protein, 9 aa, Nocardiopsis prasina
TGALPQSPT

SEQ ID NO: 30 - protein, 10 aa, Nocardiopsis prasina
TGALPQSPTP

SEQ ID NO: 31 - protein, 11 aa, Nocardiopsis prasina
TGALPQSPTPE

SEQ ID NO: 32 - protein, 12 aa, Nocardiopsis prasina
TGALPQSPTPEA

SEQ ID NO: 33 - protein, 13 aa, Nocardiopsis prasina
TGALPQSPTPEAD

SEQ ID NO: 34 - protein, 14 aa, Nocardiopsis prasina
TGALPQSPTPEADA

SEQ ID NO: 35 - protein, 15 aa, Nocardiopsis prasina
TGALPQSPTPEADAV

SEQ ID NO: 36 - protein, 16 aa, Nocardiopsis prasina
TGALPQSPTPEADAVS

SEQ ID NO: 37 - protein, 17 aa, Nocardiopsis prasina
TGALPQSPTPEADAVSM

SEQ ID NO: 38 - protein, 18 aa, Nocardiopsis prasina
TGALPQSPTPEADAVSMQ

SEQ ID NO: 39 - protein, 19 aa, Nocardiopsis prasina
TGALPQSPTPEADAVSMQE

SEQ ID NO: 40 - protein, 20 aa, Nocardiopsis prasina
TGALPQSPTPEADAVSMQEA

SEQ ID NO: 41 - protein, 21 aa, Nocardiopsis prasina
TGALPQSPTPEADAVSMQEAL

SEQ ID NO: 42 - protein, 22 aa, Nocardiopsis prasina
TGALPQSPTPEADAVSMQEALQ

SEQ ID NO: 43 - protein, 23 aa, Nocardiopsis prasina
TGALPQSPTPEADAVSMQEALQR

SEQ ID NO: 44 - protein, 24 aa, Nocardiopsis prasina
TGALPQSPTPEADAVSMQEALQRD

SEQ ID NO: 45 - protein, 25 aa, Nocardiopsis prasina
TGALPQSPTPEADAVSMQEALQRDL

SEQ ID NO: 46 - protein, 26 aa, Nocardiopsis prasina
TGALPQSPTPEADAVSMQEALQRDLD

SEQ ID NO: 47 - protein, 27 aa, Nocardiopsis prasina
TGALPQSPTPEADAVSMQEALQRDLDL

SEQ ID NO: 48 - protein, 28 aa, Nocardiopsis prasina
TGALPQSPTPEADAVSMQEALQRDLDLT

SEQ ID NO: 49 - protein, 153 aa, Bacillus licheniformis
MPYYIIALLIIGIDQFTKWLVVSKMEYGESIPVIDGFFQITSHRNTGAAWGILAGQMWFFYIITTVVIIGIVYYIQKHAKGQILLGIALGLMLGGAVGNFIDRVFRQEVVDFIHVTIVNYHYPIFNIADSSLCIGVLLLFIQMLLDGKKKKEL

SEQ ID NO: 50 - protein, 182 aa, Bacillus licheniformis
MKNSRKKEILSWVKTLVIAAALVMVCRYFLFTPSTVLGDSMYPTLEDGNMVMVSKISDIQRFDKIIFHAPDSDENYVKRVIGLPGDTIEMKDDVLYINGKAYDEPYLKKNKQKLTLHEHLTDNFTLEKLTGEQKVPEDHLFVMGDNRQNSKDSRFFGFITMDSVVGKVEFRYFPFNEIGGIE

SEQ ID NO: 51 - protein, 194 aa, Bacillus licheniformis
MKHVMKWISNFLYVIIFTIIIAAVIVVISTKSSGGEPQLFGYQLKTVLSGSMEPEFKTGSVIAVQKVENPGSLKKGDIITFMQDENTMVTHRIIGITKNKSNLMFKTKGDNNQNPDSDPVLAENVVAKYSGITVPYAGYLLDFASKPIGTAILLIVPGLLLILYAVITVSAALREIDQKAKAIEAAGKDQSVSM

SEQ ID NO: 52 - protein, 4 aa, Bacillus clausii
AEEA

SEQ ID NO: 53 - protein, 5 aa, Bacillus clausii
AEEAK

SEQ ID NO: 54 - protein, 6 aa, Bacillus clausii
AEEAKE

SEQ ID NO: 55 - protein, 7 aa, Bacillus clausii
AEEAKEK

SEQ ID NO: 56 - protein, 8 aa, Bacillus clausii
AEEAKEKY

SEQ ID NO: 57 - protein, 9 aa, Bacillus clausii
AEEAKEKYL

SEQ ID NO: 58 - protein, 10 aa, Bacillus clausii
AEEAKEKYLI

SEQ ID NO: 59 - protein, 11 aa, Bacillus clausii
AEEAKEKYLIG

SEQ ID NO: 60 - protein, 12 aa, Bacillus clausii
AEEAKEKYLIGF

SEQ ID NO: 61 - protein, 13 aa, Bacillus clausii
AEEAKEKYLIGFN

SEQ ID NO: 62 - protein, 14 aa, Bacillus clausii
AEEAKEKYLIGFNE

SEQ ID NO: 63 - protein, 15 aa, Bacillus clausii
AEEAKEKYLIGFNEQ

SEQ ID NO: 64 - protein, 16 aa, Bacillus clausii
AEEAKEKYLIGFNEQE

SEQ ID NO: 65 - protein, 17 aa, Bacillus clausii
AEEAKEKYLIGFNEQEA

SEQ ID NO: 66 - protein, 18 aa, Bacillus clausii
AEEAKEKYLIGFNEQEAV

SEQ ID NO: 67 - protein, 19 aa, Bacillus clausii
AEEAKEKYLIGFNEQEAVS

SEQ ID NO: 68 - protein, 20 aa, Bacillus clausii
AEEAKEKYLIGFNEQEAVSE

SEQ ID NO: 69 - protein, 21 aa, Bacillus clausii
AEEAKEKYLIGFNEQEAVSEF

SEQ ID NO: 70 - protein, 22 aa, Bacillus clausii
AEEAKEKYLIGFNEQEAVSEFV

SEQ ID NO: 71 - protein, 23 aa, Bacillus clausii
AEEAKEKYLIGFNEQEAVSEFVE

SEQ ID NO: 72 - protein, 24 aa, Bacillus clausii
AEEAKEKYLIGFNEQEAVSEFVEQ

SEQ ID NO: 73 - protein, 25 aa, Bacillus clausii
AEEAKEKYLIGFNEQEAVSEFVEQV

SEQ ID NO: 74 - protein, 26 aa, Bacillus clausii
AEEAKEKYLIGFNEQEAVSEFVEQVE

SEQ ID NO: 75 - protein, 27 aa, Bacillus clausii
AEEAKEKYLIGFNEQEAVSEFVEQVEA

SEQ ID NO: 76 - protein, 28 aa, Bacillus clausii
AEEAKEKYLIGFNEQEAVSEFVEQVEAN

SEQ ID NO: 77 - DNA, 1560 bp, synthetic construct
  source 1..1560: mol_type = other DNA
  misc_feature 1..21: note = SP-linker
acaggagcattaccgcagtctatgaaacaacaaaaacggctttacgcccgattgctgacgctgttatttgcgctcatcttcttgctgcctcattctgcagcagcggcggcaaatcttaatgggacgctgatgcagtattttgaatggtacatgcccaatgacggccaacattggaggcgtttgcaaaacgactcggcatatttggctgaacacggtattactgccgtctggattcccccggcatataagggaacgagccaagcggatgtgggctacggtgcttacgacctttatgatttaggggagtttcatcaaaaagggacggttcggacaaagtacggcacaaaaggagagctgcaatctgcgatcaaaagtcttcattcccgcgacattaacgtttacggggatgtggtcatcaaccacaaaggcggcgctgatgcgaccgaagatgtaaccgcggttgaagtcgatcccgctgaccgcaaccgcgtaatttcaggagaacacctaattaaagcctggacacattttcattttccggggcgcggcagcacatacagcgattttaaatggcattggtaccattttgacggaaccgattgggacgagtcccgaaagctgaaccgcatctataagtttcaaggaaaggcttgggattgggaagtttccaatgaaaacggcaactatgattatttgatgtatgccgacatcgattatgaccatcctgatgtcgcagcagaaattaagagatggggcacttggtatgccaatgaactgcaattggacggtttccgtcttgatgctgtcaaacacattaaattttcttttttgcgggattgggttaatcatgtcagggaaaaaacggggaaggaaatgtttacggtagctgaatattggcagaatgacttgggcgcgctggaaaactatttgaacaaaacaaattttaatcattcagtgtttgacgtgccgcttcattatcagttccatgctgcatcgacacagggaggcggctatgatatgaggaaattgctgaacggtacggtcgtttccaagcatccgttgaaatcggttacatttgtcgataaccatgatacacagccggggcaatcgcttgagtcgactgtccaaacatggtttaagccgcttgcttacgcttttattctcacaagggaatctggataccctcaggttttctacggggatatgtacgggacgaaaggagactcccagcgcgaaattcctgccttgaaacacaaaattgaaccgatcttaaaagcgagaaaacagtatgcgtacggagcacagcatgattatttcgaccaccatgacattgtcggctggacaagggaaggcgacagctcggttgcaaattcaggtttggcggcattaataacagacggacccggtggggcaaagcgaatgtatgtcggccggcaaaacgccggtgagacatggcatgacattaccggaaaccgttcggagccggttgtcatcaattcggaaggctggggagagtttcacgtaaacggcgggtcggtttcaatttatgttcaaagatag

SEQ ID NO: 78 - DNA, 1560 bp, synthetic construct
  source 1..1560: mol_type = other DNA
  misc_feature 1..21: note = SP-linker
gctgaagaagcaaaagaaaaaatgaaacaacaaaaacggctttacgcccgattgctgacgctgttatttgcgctcatcttcttgctgcctcattctgcagcagcggcggcaaatcttaatgggacgctgatgcagtattttgaatggtacatgcccaatgacggccaacattggaggcgtttgcaaaacgactcggcatatttggctgaacacggtattactgccgtctggattcccccggcatataagggaacgagccaagcggatgtgggctacggtgcttacgacctttatgatttaggggagtttcatcaaaaagggacggttcggacaaagtacggcacaaaaggagagctgcaatctgcgatcaaaagtcttcattcccgcgacattaacgtttacggggatgtggtcatcaaccacaaaggcggcgctgatgcgaccgaagatgtaaccgcggttgaagtcgatcccgctgaccgcaaccgcgtaatttcaggagaacacctaattaaagcctggacacattttcattttccggggcgcggcagcacatacagcgattttaaatggcattggtaccattttgacggaaccgattgggacgagtcccgaaagctgaaccgcatctataagtttcaaggaaaggcttgggattgggaagtttccaatgaaaacggcaactatgattatttgatgtatgccgacatcgattatgaccatcctgatgtcgcagcagaaattaagagatggggcacttggtatgccaatgaactgcaattggacggtttccgtcttgatgctgtcaaacacattaaattttcttttttgcgggattgggttaatcatgtcagggaaaaaacggggaaggaaatgtttacggtagctgaatattggcagaatgacttgggcgcgctggaaaactatttgaacaaaacaaattttaatcattcagtgtttgacgtgccgcttcattatcagttccatgctgcatcgacacagggaggcggctatgatatgaggaaattgctgaacggtacggtcgtttccaagcatccgttgaaatcggttacatttgtcgataaccatgatacacagccggggcaatcgcttgagtcgactgtccaaacatggtttaagccgcttgcttacgcttttattctcacaagggaatctggataccctcaggttttctacggggatatgtacgggacgaaaggagactcccagcgcgaaattcctgccttgaaacacaaaattgaaccgatcttaaaagcgagaaaacagtatgcgtacggagcacagcatgattatttcgaccaccatgacattgtcggctggacaagggaaggcgacagctcggttgcaaattcaggtttggcggcattaataacagacggacccggtggggcaaagcgaatgtatgtcggccggcaaaacgccggtgagacatggcatgacattaccggaaaccgttcggagccggttgtcatcaattcggaaggctggggagagtttcacgtaaacggcgggtcggtttcaatttatgttcaaagatag

SEQ ID NO: 79 - protein, 7 aa, Bacillus pumilus
SHDEARR

SEQ ID NO: 80 - protein, 380 aa, synthetic construct
  SIGNAL 1..27
MMKKVSGLIILSMMLLSGFYMETAYGAAEEAKEKYLIGFNEQEAVSEFVEQVEANDEVAILSEEEEVEIELLHEFETIPVLSVELSPEDVDALELDPAISYIEEDAEVTTMAQSVPWGISRVQAPAAHNRGLTGSGVKVAVLDTGISTHPDLNIRGGASFVPGEPSTQDGNGHGTHVAGTIAALNNSIGVLGVAPSAELYAVKVLGASGSGSVSSIAQGLEWAGNNGMHVANLSLGSPSPSATLEQAVNSATSRGVLVVAASGNSGAGSISYPARYANAMAVGATDQNNNRASFSQYGAGLDIVAPGVNVQSTYPGSTYASLNGTSMATPHVAGAAALVKQKNPSWSNVQIRNHLKNTATSLGSTNLYGSGLVNAEAATR

SEQ ID NO: 81 - protein, 29 aa, Bacillus licheniformis
MMRKKSFWLGMLTAFMLVFTMAFSDSASA

SEQ ID NO: 82 - DNA, 87 bp, Bacillus licheniformis
  source 1..87: mol_type = other DNA
atgatgaggaaaaagagtttttggcttgggatgctgacggccttcatgctcgtgttcacgatggcattcagcgattccgcttctgct

SEQ ID NO: 83 - protein, 4 aa, Bacillus pumilus
SHDE

SEQ ID NO: 84 - protein, 5 aa, Bacillus pumilus
SHDEA

SEQ ID NO: 85 - protein, 6 aa, Bacillus pumilus
SHDEAR

SEQ ID NO: 86 - protein, 7 aa, Bacillus pumilus
SHDEARR

SEQ ID NO: 87 - protein, 8 aa, Bacillus pumilus
SHDEARRG

SEQ ID NO: 88 - protein, 9 aa, Bacillus pumilus
SHDEARRGH

SEQ ID NO: 89 - protein, 10 aa, Bacillus pumilus
SHDEARRGHT

SEQ ID NO: 90 - protein, 11 aa, Bacillus pumilus
SHDEARRGHTA

SEQ ID NO: 91 - protein, 12 aa, Bacillus pumilus
SHDEARRGHTAS

SEQ ID NO: 92 - protein, 13 aa, Bacillus pumilus
SHDEARRGHTASI

SEQ ID NO: 93 - protein, 14 aa, Bacillus pumilus
SHDEARRGHTASIG

SEQ ID NO: 94 - protein, 15 aa, Bacillus pumilus
SHDEARRGHTASIGY

SEQ ID NO: 95 - protein, 16 aa, Bacillus pumilus
SHDEARRGHTASIGYT

SEQ ID NO: 96 - protein, 17 aa, Bacillus pumilus
SHDEARRGHTASIGYTA

SEQ ID NO: 97 - protein, 7 aa, Bacillus pumilus
TPQMEKR

SEQ ID NO: 98 - protein, 186 aa, Bacillus licheniformis; identical to SEQ ID NO: 23

SEQ ID NO: 99 - DNA, 2213 bp, synthetic construct
  misc_feature 1..2213: note = artificial sequence
  source 1..2213: mol_type = other DNA
gaaatatgtttgaaccttcttcagattacaaatatattcggacggactctacctcaaatgcttatctaactatagaatgacatacaagcacaaccttgaaaatttgaaaatataactaccaatgaacttgttcatgtgaattatcgctgtatttaattttctcaattcaatatataatatgccaatacattgttacaagtagaaattaagacacccttgatagccttactatacctaacatgatgtagtattaaatgaatatgtaaatatatttatgataagaagcgacttatttataatcattacatatttttctattggaatgattaagattccaatagaatagtgtataaattatttatcttgaaaggagggatgcctaaaaacgaagaacattaaaaacatatatttgcaccgtctaatggatttatgaaaaatcattttatcagtttgaaaattatgtattatggagctctataaaaatgaggagggaaccgaatgatgaaaaaagtaagtggcttaatcatattatcgatgatgctgttgtctggtttttatatggaaacagcttatggtgcggctgaagaagcaaaagaaaaagcaaatcttaatgggacgctgatgcagtattttgaatggtacatgcccaatgacggccaacattggaggcgtttgcaaaacgactcggcatatttggctgaacacggtattactgccgtctggattcccccggcatataagggaacgagccaagcggatgtgggctacggtgcttacgacctttatgatttaggggagtttcatcaaaaagggacggttcggacaaagtacggcacaaaaggagagctgcaatctgcgatcaaaagtcttcattcccgcgacattaacgtttacggggatgtggtcatcaaccacaaaggcggcgctgatgcgaccgaagatgtaaccgcggttgaagtcgatcccgctgaccgcaaccgcgtaatttcaggagaacacctaattaaagcctggacacattttcattttccggggcgcggcagcacatacagcgattttaaatggcattggtaccattttgacggaaccgattgggacgagtcccgaaagctgaaccgcatctataagtttcaaggaaaggcttgggattgggaagtttccaatgaaaacggcaactatgattatttgatgtatgccgacatcgattatgaccatcctgatgtcgcagcagaaattaagagatggggcacttggtatgccaatgaactgcaattggacggtttccgtcttgatgctgtcaaacacattaaattttcttttttgcgggattgggttaatcatgtcagggaaaaaacggggaaggaaatgtttacggtagctgaatattggcagaatgacttgggcgcgctggaaaactatttgaacaaaacaaattttaatcattcagtgtttgacgtgccgcttcattatcagttccatgctgcatcgacacagggaggcggctatgatatgaggaaattgctgaacggtacggtcgtttccaagcatccgttgaaatcggttacatttgtcgataaccatgatacacagccggggcaatcgcttgagtcgactgtccaaacatggtttaagccgcttgcttacgcttttattctcacaagggaatctggataccctcaggttttctacggggatatgtacgggacgaaaggagactcccagcgcgaaattcctgccttgaaacacaaaattgaaccgatcttaaaagcgagaaaacagtatgcgtacggagcacagcatgattatttcgaccaccatgacattgtcggctggacaagggaaggcgacagctcggttgcaaattcaggtttggcggcattaataacagacggacccggtggggcaaagcgaatgtatgtcggccggcaaaacgccggtgagacatggcatgacattaccggaaaccgttcggagccggttgtcatcaattcggaaggctggggagagtttcacgtaaacggcgggtcggtttcaatttatgttcaaagatagacgcgtagggcccgcggctagcggccgcgtcgactagaagagcagagaggacggatttcctgaaggaaatccgtttttttattttgcccgtcttataaatttcgttgttcaataatcgcatccgattgcagtataaatttaacgatcactcatcatgttca

SEQ ID NO: 100 - DNA, 1827 bp, synthetic construct
  misc_feature 1..1827: note = artificial sequence
  source 1..1827: mol_type = other DNA
gaaatatgtttgaaccttcttcagattacaaatatattcggacggactctacctcaaatgcttatctaactatagaatgacatacaagcacaaccttgaaaatttgaaaatataactaccaatgaacttgttcatgtgaattatcgctgtatttaattttctcaattcaatatataatatgccaatacattgttacaagtagaaattaagacacccttgatagccttactatacctaacatgatgtagtattaaatgaatatgtaaatatatttatgataagaagcgacttatttataatcattacatatttttctattggaatgattaagattccaatagaatagtgtataaattatttatcttgaaaggagggatgcctaaaaacgaagaacattaaaaacatatatttgcaccgtctaatggatagaaaggaggtgatccagccgcaccttatgaaaaatcattttatcagtttgaaaattatgtattatggagctcagaggaggagagtgagtaatgatgaggaaaaagagtttttggcttgggatgctgacggccttcatgctcgtgttcacgatggcattcagcgattccgcttctgctgctgaagaagcaaaagaaaaatatttaattggctttaatgagcaggaagctgtcagtgagtttgtagaacaagtagaggcaaatgacgaggtcgccattctctctgaggaagaggaagtcgaaattgaattgcttcatgaatttgaaacgattcctgttttatccgttgagttaagcccagaagatgtggacgcgcttgaactcgatccagcgatttcttatattgaagaggatgcagaagtaacgacaatggcgcaatcagtgccatggggaattagccgtgtgcaagccccagctgcccataaccgtggattgacaggttctggtgtaaaagttgctgtcctcgatacaggtatttccactcatccagacttaaatattcgtggtggcgctagctttgtaccaggggaaccatccactcaagatgggaatgggcatggcacgcatgtggccgggacgattgctgctttaaacaattcgattggcgttcttggcgtagcgccgagcgcggaactatacgctgttaaagtattaggggcgagcggttcaggttcggtcagctcgattgcccaaggattggaatgggcagggaacaatggcatgcacgttgctaatttgagtttaggaagcccttcgccaagtgccacacttgagcaagctgttaatagcgcgacttctagaggcgttcttgttgtagcggcatctgggaattcaggtgcaggctcaatcagctatccggcccgttatgcgaacgcaatggcagtcggagctactgaccaaaacaacaaccgcgccagcttttcacagtatggcgcagggcttgacattgtcgcaccaggtgtaaacgtgcagagcacatacccaggttcaacgtatgccagcttaaacggtacatcgatggctactcctcatgttgcaggtgcagcagcccttgttaaacaaaagaacccatcttggtccaatgtacaaatccgcaatcatctaaagaatacggcaacgagcttaggaagcacgaacttgtatggaagcggacttgtcaatgcagaagcggcaacgcgataacgcgtagggcccgcggctagcggccgcgtcgactagaagagcagagaggacggatttcctgaaggaaatccgtttttttattttgcccgtcttataaatttcgttgttcaataatcgcatccgattgcagtataaatttaacgatcactcatcatgttca

SEQ ID NO: 101 - protein, 4 aa, Bacillus pumilus
TPQM

SEQ ID NO: 102 - protein, 5 aa, Bacillus pumilus
TPQME

SEQ ID NO: 103 - protein, 6 aa, Bacillus pumilus
TPQMEK

SEQ ID NO: 104 - protein, 7 aa, Bacillus pumilus
TPQMEKR

SEQ ID NO: 105 - protein, 8 aa, Bacillus pumilus
TPQMEKRP

SEQ ID NO: 106 - protein, 9 aa, Bacillus pumilus
TPQMEKRPV

SEQ ID NO: 107 - protein, 10 aa, Bacillus pumilus
TPQMEKRPVM

SEQ ID NO: 108 - protein, 11 aa, Bacillus pumilus
TPQMEKRPVMH

SEQ ID NO: 109 - protein, 12 aa, Bacillus pumilus
TPQMEKRPVMHQ

SEQ ID NO: 110 - protein, 13 aa, Bacillus pumilus
TPQMEKRPVMHQV

SEQ ID NO: 111 - protein, 14 aa, Bacillus pumilus
TPQMEKRPVMHQVK

SEQ ID NO: 112 - protein, 15 aa, Bacillus pumilus
TPQMEKRPVMHQVKL

SEQ ID NO: 113 - protein, 16 aa, Bacillus pumilus
TPQMEKRPVMHQVKLT

SEQ ID NO: 114 - protein, 17 aa, Bacillus pumilus
TPQMEKRPVMHQVKLTT

SEQ ID NO: 115 - protein, 18 aa, Bacillus pumilus
TPQMEKRPVMHQVKLTTE

SEQ ID NO: 116 - protein, 19 aa, Bacillus pumilus
TPQMEKRPVMHQVKLTTEQ

SEQ ID NO: 117 - protein, 20 aa, Bacillus pumilus
TPQMEKRPVMHQVKLTTEQQ

SEQ ID NO: 118 - protein, 21 aa, Bacillus pumilus
TPQMEKRPVMHQVKLTTEQQK

SEQ ID NO: 119 - protein, 22 aa, Bacillus pumilus
TPQMEKRPVMHQVKLTTEQQKQ

SEQ ID NO: 120 - protein, 23 aa, Bacillus pumilus
TPQMEKRPVMHQVKLTTEQQKQI

SEQ ID NO: 121 - protein, 24 aa, Bacillus pumilus
TPQMEKRPVMHQVKLTTEQQKQIE

SEQ ID NO: 122 - protein, 25 aa, Bacillus pumilus
TPQMEKRPVMHQVKLTTEQQKQIEM

SEQ ID NO: 123 - protein, 26 aa, Bacillus pumilus
TPQMEKRPVMHQVKLTTEQQKQIEML

SEQ ID NO: 124 - protein, 27 aa, Bacillus pumilus
TPQMEKRPVMHQVKLTTEQQKQIEMLE

SEQ ID NO: 125 - protein, 28 aa, Bacillus pumilus
TPQMEKRPVMHQVKLTTEQQKQIEMLEQ

SEQ ID NO: 126 - protein, 29 aa, Bacillus pumilus
TPQMEKRPVMHQVKLTTEQQKQIEMLEQQ

SEQ ID NO: 127 - DNA, 1801 bp, synthetic construct
  misc_feature 1..1801: note = artificial sequence
  source 1..1801: mol_type = other DNA
gaaatatgtttgaaccttcttcagattacaaatatattcggacggactctacctcaaatgcttatctaactatagaatgacatacaagcacaaccttgaaaatttgaaaatataactaccaatgaacttgttcatgtgaattatcgctgtatttaattttctcaattcaatatataatatgccaatacattgttacaagtagaaattaagacacccttgatagccttactatacctaacatgatgtagtattaaatgaatatgtaaatatatttatgataagaagcgacttatttataatcattacatatttttctattggaatgattaagattccaatagaatagtgtataaattatttatcttgaaaggagggatgcctaaaaacgaagaacattaaaaacatatatttgcaccgtctaatggatttatgaaaaatcattttatcagtttgaaaattatgtattatggagctctataaaaatgaggagggaaccgaatgaaatttaaaacgttatcagtagtattcgtgatgattagtgtcataagtgttgttagttattttacgtcagaagtgacagcgacaggagcattaccgcagtctccgacaccggaagcagatgcagtctcaatgcaagaagcactgcaaagagatcttgatcttacatcagcagaagcagaagaacttcttgctgcacaagatacagcatttgaagtggatgaagcagcggcagaagcagcaggagatgcatatggcggctcagtttttgatacagaatcacttgaacttacggttcttgttacagatgcagcagcagttgaagcagttgaagcaacaggagcaggaacagaacttgtttcatatggaattgatggccttgatgaaattgttcaagaactgaatgcagctgatgctgttccgggcgttgttggctggtatccggatgttgctggagatacagttgtccttgaagttcttgaaggatcaggcgcagatgtttcaggcctgctggcagatgcaggagtcgatgcatcagcagttgaagttacaacatcagatcaaccggaactttatgcagatattattggcggcctggcatatacaatgggcggcagatgcagcgttggctttgcagcaacaaatgcagcaggccaaccgggctttgttacagcaggccattgcggcagagttggcacacaggttacaattggcaatggcagaggcgtttttgaacaaagcgtttttccgggcaatgatgcagcatttgttagaggcacatcaaattttacacttacaaatctggtttcaagatataatacaggcggctatgcaacagttgcaggccataatcaagcaccgattggctcatcagtttgcagatcaggctcaacaacaggctggcattgcggcacaattcaagcaagaggccaaagcgttagctatccggaaggcacagttacaaatatgacaagaacaacagtttgtgcagaaccgggcgattcaggcggctcatatattagcggcacacaagcacaaggcgttacatcaggcggctcaggcaattgcagaacaggcggcacaacattttaccaagaagttacaccgatggttaattcatggggcgttagacttagaacataacgcgtagggcccgcggctagcggccgcgtcgactagaagagcagagaggacggatttcctgaaggaaatccgtttttttattttgcccgtcttataaatttcgttgttcaataatcgcatccgattgcagtataaatttaacgatcactcatcatgttca

SEQ ID NO: 128 - DNA, 3934 bp, synthetic construct
  misc_feature 1..3934: note = artificial sequence
  source 1..3934: mol_type = other DNA
gtgaaggttccgcatgatatgccgaatcttccggtggcgcgcgtactttggaagcctcagccgtctctgagaacatcggctgaagcgtggattttggctggcggtgctcaccatacatgcctttcgtaccagctgacagccgagcagatgctcgattgggccgaaatgtcgggcattgaagcggtgttgatcaatcgtgatacaacgattttaaatcttcgcaatgaactcaaatggagtgaagctgcatatcggcttcgcaagttttaagggggtgaggacttatcccttacacaatcggagttgactttggaacattgtcagggcgtgcagttctcgtcgatgtccggacaggtgaggaaatcgcgacagctgtcaaagagtacacgcacggggtgatagaccgggagcttccggtctcaaagcgaaagcttccgagagactgggcgctccagcatccggccgattacattgaagtgctggaggaaacgattccgagccttttgaaacagtcaaaagcggatccgaaagaaatcatcggaatcggaatcgatttcacggcttgcacgattttgcccgttgacgagaacgggactcctctttgtatgagggaagagtatgcgtcagaaccgcacagctatgtgaagctttggaagcaccatgctgcacaggagcaggcgaatcgcttaaatcaaatcgcggaagaaagaaatgaaccttttcttcaaacatacggcgggaaaatttcttccgagtggctcgttccaaaagtgatgcaaatcgcggaagaagcgcctgacatttatgatgccgcagccgagatcatggaagcggccgactggatcgtctatatgctgtgcggaaccagaaagcgcaacaattgcacagcgggttataaagcgatttggaacaataagagcggctatccttccgacgatttcttcgcaagcctgcatccgaagctgaaaaatatcgttcgggaaaaactaacggaggatatttattctgtaggcgaaaaagcgggcggactgactgaagaaatggccgggaagacagggcttctggcaggtacggcggtcgctgtcgcaaatgttgatgctcatgtgtcggttccggcggtcggcatcacagagccgggcaagatgctgatgatcatgggaacgtctacctgtcacatgctgctcggcgaggatgtcaggatggtgccgggaatgtgcggcgtcgttgaagacgggattctgccgggctatgtcggctatgaagcgggccaatcgtgcgttggcgaccattttcattggctgattcaacactttgttccagaagcgtatttgaaagaagctgaagccgaagggatttccatttacgaactgctgtctcaaaaggccggcagtctccaaatcggtgaaagcggtttgcttgcattggattggtggaacggaaaccgttcaacactcgttgatgccgatctgacgggaatgctgctcggtatgacccttgccactaagcctgaagagatataccgtgcattggttgaagcgactgcctgcgggacgaggatcattattgaaacgttcagacaaagcggcgtgccgatcgaggagctgtatgccgcaggaggaatcgccgaaaaaaatccgtttatcatgcaggtttacgcggatgtcaccaacatggaaatcaaaatttccggatctccgcaggcgccggctttaggttcagcgatattcggagcgctcgcggccggaagcatgaacggcggttacgaccatatcgaagaagcagtcgcacatatgggcaagatcaaggataaaacgtacaaaccaattcctgaaaacgtttccttatacgatcagctttatgcggaatataaggagctttacacgtacttcggaaagcaaaacaatgtgatgaaacgccttaaaaaattgaaaaacatccagtcccttagttctgaccccggtaaagcgatggcttagagggaggagaaaactgtgctggaatctttgaaagaacaagtattaaaagcgaatttgcagcttgaagaataccggcttgtcacctttacatggggaaatgtcagcggtattgaccgggagaataagctggtcgtcatcaagccgagcggtgtcaaatacagcgatttgaaagccgaagatttagtggttctgaatatggacggcgagattgtggaaggggatctgaagccatcttccgatacgccgacacacctctatctttaccggcagtttcaatcgatcggcgggatcgtccatacgcattccccgtgggcgacaagctgggctcagtcagggaaggacattccgtcgctcggaacgactcatgccgactactaccacggcgacattccgtgtacacgggaaatggatcccgatgaaatcaggagtcaatacgagctgaatacaggaaaagtgattgtagagacgttccggcatcttgaccccctggcggtgcccgccgttctcgtgaacaatcacgggccgttttgctggggaaaagacgccttaactgccgtacacaatgccgtcgtcctggaagaagtcgccaagatggcgtaccgctccctgatgctgaatccgtctcttaagcggattaagagcgctttgcaggataagcattattttcgaaagcacggggcagacgcctattacggccaatagaggagggaagctgccaatgaatgacttgatctcttatgtgaaaaaaactttgggcgcatgcgaatgcggaaccgtccaccacccgcttacagtcgaaaaaatcgcgatcggcgacaatgctgttgagcaagagctgcccgctttcgtgaaatcggcttcctataaaaaagccgctgtcatttatgatgaaacgaccggacggttagccggcaagcggattgcctctcttcttgaggaaacggctgaaacggttccggtgctgctggaagctaatgaagcgggcgatgtgacggcggatgagcaaacattggtgagtgcattgatcggtgtaccgattgatgcggatgtactaattgcggccggagcgggcacgattcacgacatcgtcaggttttgcgcctatcagcgcggcattccgtttatttcagttcctacggctccgtcggttgacggttttacttcagccggcgcaccgctgattttaaaaggaaagaaacagacggttcaaacgacagcgccgatcgcgctttttgccgatttggagctcttgtgtcaagcgccgcagaacatggtagccgcaggttttggcgatatgctcggcaaggtgacgtcgcttgcggattgggagatttcccgcttgcttgccggcgagccgtattgtccggccgccagccggctcacgagggaagcgcttgatcaatgtcttgaccgcaacgttcgcagatgctgctgaagagattattaaaaagctgaaagcaaaaggctatcaattggtaactgtatctcagcttgaagaagtgaagaagcagagaggctattgaataaatgagtagaaagcgccatatcggcgcttttcttttggaagaaaatatagggaaaatggtacttgttaaaaattcggaatatttatacaatatcatatgtatcacattgaaaggaggggcctgctgtccagactgtccgctgtgtaaaaaaaaggaataaaggggggttgacattattttactgatatgtataatataatttgtataagaaaatggaggggccctcgaaacgtaagatgaaaccttagataaaagtgctttttttgttgcaattgaagaattattaatgttaagcttaattaaagataatatctttgaattgtaacgcccctcaaaagtaagaactacaaaaaaagaatacgttatatagaaatatgtttgaaccttcttcagattacaaatatattcggacggactctacctcaaatgctt

SEQ ID NO: 129 - DNA, 4368 bp, synthetic construct
  misc_feature 1..4368: note = artificial sequence
  source 1..4368: mol_type = other DNA
ttcaataatcgcatccgattgcagtataaatttaacgatcactcatcatgttcatatttatcagagctcgtgctataattatactaattttataaggaggaaaaaatatgggcatttttagtatttttgtaatcagcacagttcattatcaaccaaacaaaaaataagtggttataatgaatcgttaataagcaaaattcatataaccaaattaaagagggttataatgaacgagaaaaatataaaacacagtcaaaactttattacttcaaaacataatatagataaaataatgacaaatataagattaaatgaacatgataatatctttgaaatcggctcaggaaaaggccattttacccttgaattagtaaagaggtgtaatttcgtaactgccattgaaatagaccataaattatgcaaaactacagaaaataaacttgttgatcacgataatttccaagttttaaacaaggatatattgcagtttaaatttcctaaaaaccaatcctataaaatatatggtaatataccttataacataagtacggatataatacgcaaaattgtttttgatagtatagctaatgagatttatttaatcgtggaatacgggtttgctaaaagattattaaatacaaaacgctcattggcattacttttaatggcagaagttgatatttctatattaagtatggttccaagagaatattttcatcctaaacctaaagtgaatagctcacttatcagattaagtagaaaaaaatcaagaatatcacacaaagataaacaaaagtataattatttcgttatgaaatgggttaacaaagaatacaagaaaatatttacaaaaaatcaatttaacaattccttaaaacatgcaggaattgacgatttaaacaatattagctttgaacaattcttatctcttttcaatagctataaattatttaataagtaagttaagggatgcataaactgcatcccttaacttgtttttcgtgtgcctattttttgtgaatcgattatgtcttttgcgcagatgctggttctcgaccattcaaggccggcttccggcggcgagcaccatctttcccactaccttgaaatgaaagcgctggagaacaataagcggcaagtgctccacggtgctaaagtcggctgcagcgcgattatgctgactgacatttaccgatctcttatcggtgcaagcctgggtgatcaacacgctgagcaagcgattcgctccgtttatgaaaagctccctgacggtaagaaaatggcagagtggatgaggcgtatcggcgggcctgtatcattcaaagaactcgatgttgaagaagagctggtgagagaagcgctcgcatacgcccatcagctcagagaccggtatacgggactgaaaatcatcaatcaatacggccttttgccggggcttttaggcaaaggaccaggcgtgaaaggggttaaaatgtgaaaaggttcctttcatctatctttatggtcacggtcgctgtatgtttgcttttatcggggtgcaaggcgagtcctgcctccgatcaagcggacggcaccgaactgacattttggacattcaacggccttcatgaacagttttatgctgagatggtgaaagaatggaacaaaaagtatcccgagcgaaaaatcaaattaaatacagtggtgtatccgtatggacagatgcatgacaatttatctatctcgcttttagccgggaaaggggttccagatattgccgatgttgagctggggcgctattcgaactttttgaagggctctgacattcctcttaccgatttaacgccgcttgtggaggacgaacgcgacaagtttgttgaagcgaggctgacgctctacagcaagaacggcaagctttacggacttgacacacatgtcggaactaccgtgatgtattacaacatggaaatgatgaataaagcaggcgttgatccggacgacatcaaaacatgggaagattacagggaagcgggcaaaaaggtcgtcaaagctctcggaaagccgatgacgacgattgaaacgaccgacccgaattcatttctgccgctggtttcccagcagggatccggttactttgatgagcaggggcggttgacattaaacaatgagacaaacgtgaaaacgctcgaatttttaaagactttaattgagaaagacaaaattgccgtcacaacgcccggaggcaatcatcacagtgaagagtattacggatttatgaaccaaggcggcgcggcgtctgtcttaatgccgatctggtatatgggccgttttttggattatatgcctgacttgaaagggaaaatcgcgatcagaccgctgccggcatgggaagaagggggagaccgctcagcgggaatgggcggaacggccaccgtgattccaaaacaggcgaaacaggtcgatctggccaaggatttcttgaaatttgccaaagcgtcaaaagaaggcaacaccaagctgtggaccgtgctcgggttcgatccgctcagatgggatgtgtgggactcggacgaattgaaaaaaacaaatcaatatacagaatactttcaaaacggacaacacatcttttccgtgcttcttgacataaaggatgagatcaatccgctttaccttactgaggattatgcgaagacttccgatctcgtcaacagaaacatactgtacgaagcgctcaaaacgaagagcaaaacaccgaaagaagcattggacaaagcagcagctgaagtgaaagggcaatagtctttcattactgtaaagcgaggcgataacttgaagactgttaaaacagatacagtgcattcgtttccgccggtgagcagaaaaagaaagatcagacgtttattatattcagcaaaagccgcaccctacatttttacagcaccttttgtactctccttttgcatattttttctttatccgcttatcagcgtcgtcatcatgagttttcaaagcattctccccggggaagtccgcttcatcgggacggagaactataaagcattaaacaatcctacattttataccgcactattcaacaccgtaaaatacaccttttggacattgctgattttaatacctgttcctcttattctggcagtctttttagattctaaactcgtaaagtttaaaaacgtgttcaaatcggctttattcatcccggctctgacttcaaccattgtggcggggattattttcaggctgatttttggagaaatggatacatccctggcgaattcgatattggctaagctcggaggttcgccgtacaactggctgaacaatgaacataccggcatgtttttaatggtgatgctcgcatcttggagatggatggggatcaatgtcctgtactttttggcgggcttgcagaacgttccgaaagaattgtatgaagctgccgaaatcgacggggcaggcacgttcaagaagttttaccatattacgcttccgtttttaaagcccgtcagcgtctacgtgctgacgatcagcatcatcggcggcttccggatgtttgaagaaagctacgtgctgtggcagaacaactctccgggcaacatcggcctgacgatggtcggatacatttatcagcaggggcttgcctacaacaacatgggctacggatcggcgctcggcatcgtgctcttgatcatcattttcatctgcagcctcatttcattaaagctgtctggatcttttaaaaaggagggctattaatgcgtcctgccggaggcctcaacattgcgaaagtagctctgtttctgctgtttgcgatattaagctttttgtttgtgtttccgctcttctgccttgtactcggctcgctcaagccatcttcggaattgctgcgcttcggcctgaatttaaagctgagccctgaaatcctgagccttgacaattacacttacttgtttaacggaggcagcatttattttcaatggttttcgaacagcttgattctcgtggtgatatccaccgtgctgacgctcttgttttcttcaatggtcggatacgggcttgccgtctacgactttaaaggaaaaaatctcttgttcgtagccgtgctcctgatcatgatggtgccgatcgaaattctcatgctgcctttatttaaaatgacggtttctcttcatattgtcgacacatacgccggtgtgatcctgccgtttatcgtctcgcctgtagccgtgtttttcttcagacagtatgcgctcggcctgccgagagatttgcttgattccgcgagaatggacggctgcacagagttcggcatttacttcaggatcatggcgcccttgatgaagccggcatttggagcgatgatcattcttc

SEQ ID NO: 130 - DNA, 49 bp, synthetic construct
  misc_feature 1..49: note = artificial sequence
  source 1..49: mol_type = other DNA
gcatttggagcgatgatcattcttcgtgaaggttccgcatgatatgccg

SEQ ID NO: 131 - DNA, 23 bp, synthetic construct
  misc_feature 1..23: note = artificial sequence
  source 1..23: mol_type = other DNA
aagcatttgaggtagagtccgtc

SEQ ID NO: 132 - DNA, 24 bp, synthetic construct
  misc_feature 1..24: note = artificial sequence
  source 1..24: mol_type = other DNA
ttcaataatcgcatccgattgcag

SEQ ID NO: 133 - DNA, 49 bp, synthetic construct
  misc_feature 1..49: note = artificial sequence
  source 1..49: mol_type = other DNA
cggcatatcatgcggaaccttcacgaagaatgatcatcgctccaaatgc

SEQ ID NO: 134 - DNA, 1821 bp, synthetic construct
  misc_feature 1..1821: note = artificial sequence
  source 1..1821: mol_type = other DNA
gaaatatgtttgaaccttcttcagattacaaatatattcggacggactctacctcaaatgcttatctaactatagaatgacatacaagcacaaccttgaaaatttgaaaatataactaccaatgaacttgttcatgtgaattatcgctgtatttaattttctcaattcaatatataatatgccaatacattgttacaagtagaaattaagacacccttgatagccttactatacctaacatgatgtagtattaaatgaatatgtaaatatatttatgataagaagcgacttatttataatcattacatatttttctattggaatgattaagattccaatagaatagtgtataaattatttatcttgaaaggagggatgcctaaaaacgaagaacattaaaaacatatatttgcaccgtctaatggatagaaaggaggtgatccagccgcaccttatgaaaaatcattttatcagtttgaaaattatgtattatggagctcagaggaggagagtgagtaatgatgaaaaaagtaagtggcttaatcatattatcgatgatgctgttgtctggtttttatatggaaacagcttatggtgcggctgaagaagcaaaagaaaaatatttaattggctttaatgagcaggaagctgtcagtgagtttgtagaacaagtagaggcaaatgacgaggtcgccattctctctgaggaagaggaagtcgaaattgaattgcttcatgaatttgaaacgattcctgttttatccgttgagttaagcccagaagatgtggacgcgcttgaactcgatccagcgatttcttatattgaagaggatgcagaagtaacgacaatggcgcaatcagtgccatggggaattagccgtgtgcaagccccagctgcccataaccgtggattgacaggttctggtgtaaaagttgctgtcctcgatacaggtatttccactcatccagacttaaatattcgtggtggcgctagctttgtaccaggggaaccatccactcaagatgggaatgggcatggcacgcatgtggccgggacgattgctgctttaaacaattcgattggcgttcttggcgtagcgccgagcgcggaactatacgctgttaaagtattaggggcgagcggttcaggttcggtcagctcgattgcccaaggattggaatgggcagggaacaatggcatgcacgttgctaatttgagtttaggaagcccttcgccaagtgccacacttgagcaagctgttaatagcgcgacttctagaggcgttcttgttgtagcggcatctgggaattcaggtgcaggctcaatcagctatccggcccgttatgcgaacgcaatggcagtcggagctactgaccaaaacaacaaccgcgccagcttttcacagtatggcgcagggcttgacattgtcgcaccaggtgtaaacgtgcagagcacatacccaggttcaacgtatgccagcttaaacggtacatcgatggctactcctcatgttgcaggtgcagcagcccttgttaaacaaaagaacccatcttggtccaatgtacaaatccgcaatcatctaaagaatacggcaacgagcttaggaagcacgaacttgtatggaagcggacttgtcaatgcagaagcggcaacgcgataacgcgtagggcccgcggctagcggccgcgtcgactagaagagcagagaggacggatttcctgaaggaaatccgtttttttattttgcccgtcttataaatttcgttgttcaataatcgcatccgattgcagtataaatttaacgatcactcatcatgttca

SEQ ID NO: 135 - DNA, 2195 bp, synthetic construct
  misc_feature 1..2195: note = artificial sequence
  source 1..2195: mol_type = other DNA
gaaatatgtttgaaccttcttcagattacaaatatattcggacggactctacctcaaatgcttatctaactatagaatgacatacaagcacaaccttgaaaatttgaaaatataactaccaatgaacttgttcatgtgaattatcgctgtatttaattttctcaattcaatatataatatgccaatacattgttacaagtagaaattaagacacccttgatagccttactatacctaacatgatgtagtattaaatgaatatgtaaatatatttatgataagaagcgacttatttataatcattacatatttttctattggaatgattaagattccaatagaatagtgtataaattatttatcttgaaaggagggatgcctaaaaacgaagaacattaaaaacatatatttgcaccgtctaatggatttatgaaaaatcattttatcagtttgaaaattatgtattatggagctctataaaaatgaggagggaaccgaatgaaatttaaaacgttatcagtagtattcgtgatgattagtgtcataagtgttgttagttattttacgtcagaagtgacagcggcaaatcttaatgggacgctgatgcagtattttgaatggtacatgcccaatgacggccaacattggaggcgtttgcaaaacgactcggcatatttggctgaacacggtattactgccgtctggattcccccggcatataagggaacgagccaagcggatgtgggctacggtgcttacgacctttatgatttaggggagtttcatcaaaaagggacggttcggacaaagtacggcacaaaaggagagctgcaatctgcgatcaaaagtcttcattcccgcgacattaacgtttacggggatgtggtcatcaaccacaaaggcggcgctgatgcgaccgaagatgtaaccgcggttgaagtcgatcccgctgaccgcaaccgcgtaatttcaggagaacacctaattaaagcctggacacattttcattttccggggcgcggcagcacatacagcgattttaaatggcattggtaccattttgacggaaccgattgggacgagtcccgaaagctgaaccgcatctataagtttcaaggaaaggcttgggattgggaagtttccaatgaaaacggcaactatgattatttgatgtatgccgacatcgattatgaccatcctgatgtcgcagcagaaattaagagatggggcacttggtatgccaatgaactgcaattggacggtttccgtcttgatgctgtcaaacacattaaattttcttttttgcgggattgggttaatcatgtcagggaaaaaacggggaaggaaatgtttacggtagctgaatattggcagaatgacttgggcgcgctggaaaactatttgaacaaaacaaattttaatcattcagtgtttgacgtgccgcttcattatcagttccatgctgcatcgacacagggaggcggctatgatatgaggaaattgctgaacggtacggtcgtttccaagcatccgttgaaatcggttacatttgtcgataaccatgatacacagccggggcaatcgcttgagtcgactgtccaaacatggtttaagccgcttgcttacgcttttattctcacaagggaatctggataccctcaggttttctacggggatatgtacgggacgaaaggagactcccagcgcgaaattcctgccttgaaacacaaaattgaaccgatcttaaaagcgagaaaacagtatgcgtacggagcacagcatgattatttcgaccaccatgacattgtcggctggacaagggaaggcgacagctcggttgcaaattcaggtttggcggcattaataacagacggacccggtggggcaaagcgaatgtatgtcggccggcaaaacgccggtgagacatggcatgacattaccggaaaccgttcggagccggttgtcatcaattcggaaggctggggagagtttcacgtaaacggcgggtcggtttcaatttatgttcaaagatagacgcgtagggcccgcggctagcggccgcgtcgactagaagagcagagaggacggatttcctgaaggaaatccgtttttttattttgcccgtcttataaatttcgttgttcaataatcgcatccgattgcagtataaatttaacgatcactcatcatgttca

SEQ ID NO: 136 - DNA, 2216 bp, synthetic construct
  misc_feature 1..2216: note = artificial sequence
  source 1..2216: mol_type = other DNA
gaaatatgtttgaaccttcttcagattacaaatatattcggacggactctacctcaaatgcttatctaactatagaatgacatacaagcacaaccttgaaaatttgaaaatataactaccaatgaacttgttcatgtgaattatcgctgtatttaattttctcaattcaatatataatatgccaatacattgttacaagtagaaattaagacacccttgatagccttactatacctaacatgatgtagtattaaatgaatatgtaaatatatttatgataagaagcgacttatttataatcattacatatttttctattggaatgattaagattccaatagaatagtgtataaattatttatcttgaaaggagggatgcctaaaaacgaagaacattaaaaacatatatttgcaccgtctaatggatttatgaaaaatcattttatcagtttgaaaattatgtattatggagctctataaaaatgaggagggaaccgaatgaaatttaaaacgttatcagtagtattcgtgatgattagtgtcataagtgttgttagttattttacgtcagaagtgacagcgacaggagcattaccgcagtctgcaaatcttaatgggacgctgatgcagtattttgaatggtacatgcccaatgacggccaacattggaggcgtttgcaaaacgactcggcatatttggctgaacacggtattactgccgtctggattcccccggcatataagggaacgagccaagcggatgtgggctacggtgcttacgacctttatgatttaggggagtttcatcaaaaagggacggttcggacaaagtacggcacaaaaggagagctgcaatctgcgatcaaaagtcttcattcccgcgacattaacgtttacggggatgtggtcatcaaccacaaaggcggcgctgatgcgaccgaagatgtaaccgcggttgaagtcgatcccgctgaccgcaaccgcgtaatttcaggagaacacctaattaaagcctggacacattttcattttccggggcgcggcagcacatacagcgattttaaatggcattggtaccattttgacggaaccgattgggacgagtcccgaaagctgaaccgcatctataagtttcaaggaaaggcttgggattgggaagtttccaatgaaaacggcaactatgattatttgatgtatgccgacatcgattatgaccatcctgatgtcgcagcagaaattaagagatggggcacttggtatgccaatgaactgcaattggacggtttccgtcttgatgctgtcaaacacattaaattttcttttttgcgggattgggttaatcatgtcagggaaaaaacggggaaggaaatgtttacggtagctgaatattggcagaatgacttgggcgcgctggaaaactatttgaacaaaacaaattttaatcattcagtgtttgacgtgccgcttcattatcagttccatgctgcatcgacacagggaggcggctatgatatgaggaaattgctgaacggtacggtcgtttccaagcatccgttgaaatcggttacatttgtcgataaccatgatacacagccggggcaatcgcttgagtcgactgtccaaacatggtttaagccgcttgcttacgcttttattctcacaagggaatctggataccctcaggttttctacggggatatgtacgggacgaaaggagactcccagcgcgaaattcctgccttgaaacacaaaattgaaccgatcttaaaagcgagaaaacagtatgcgtacggagcacagcatgattatttcgaccaccatgacattgtcggctggacaagggaaggcgacagctcggttgcaaattcaggtttggcggcattaataacagacggacccggtggggcaaagcgaatgtatgtcggccggcaaaacgccggtgagacatggcatgacattaccggaaaccgttcggagccggttgtcatcaattcggaaggctggggagagtttcacgtaaacggcgggtcggtttcaatttatgttcaaagatagacgcgtagggcccgcggctagcggccgcgtcgactagaagagcagagaggacggatttcctgaaggaaatccgtttttttattttgcccgtcttataaatttcgttgttcaataatcgcatccgattgcagtataaatttaacgatcactcatcatgttca

SEQ ID NO: 137 - DNA, 2192 bp, synthetic construct
  misc_feature 1..2192: note = artificial sequence
  source 1..2192: mol_type = other DNA
gaaatatgtttgaaccttcttcagattacaaatatattcggacggactctacctcaaatgcttatctaactatagaatgacatacaagcacaaccttgaaaatttgaaaatataactaccaatgaacttgttcatgtgaattatcgctgtatttaattttctcaattcaatatataatatgccaatacattgttacaagtagaaattaagacacccttgatagccttactatacctaacatgatgtagtattaaatgaatatgtaaatatatttatgataagaagcgacttatttataatcattacatatttttctattggaatgattaagattccaatagaatagtgtataaattatttatcttgaaaggagggatgcctaaaaacgaagaacattaaaaacatatatttgcaccgtctaatggatttatgaaaaatcattttatcagtttgaaaattatgtattatggagctctataaaaatgaggagggaaccgaatgatgaaaaaagtaagtggcttaatcatattatcgatgatgctgttgtctggtttttatatggaaacagcttatggtgcggcaaatcttaatgggacgctgatgcagtattttgaatggtacatgcccaatgacggccaacattggaggcgtttgcaaaacgactcggcatatttggctgaacacggtattactgccgtctggattcccccggcatataagggaacgagccaagcggatgtgggctacggtgcttacgacctttatgatttaggggagtttcatcaaaaagggacggttcggacaaagtacggcacaaaaggagagctgcaatctgcgatcaaaagtcttcattcccgcgacattaacgtttacggggatgtggtcatcaaccacaaaggcggcgctgatgcgaccgaagatgtaaccgcggttgaagtcgatcccgctgaccgcaaccgcgtaatttcaggagaacacctaattaaagcctggacacattttcattttccggggcgcggcagcacatacagcgattttaaatggcattggtaccattttgacggaaccgattgggacgagtcccgaaagctgaaccgcatctataagtttcaaggaaaggcttgggattgggaagtttccaatgaaaacggcaactatgattatttgatgtatgccgacatcgattatgaccatcctgatgtcgcagcagaaattaagagatggggcacttggtatgccaatgaactgcaattggacggtttccgtcttgatgctgtcaaacacattaaattttcttttttgcgggattgggttaatcatgtcagggaaaaaacggggaaggaaatgtttacggtagctgaatattggcagaatgacttgggcgcgctggaaaactatttgaacaaaacaaattttaatcattcagtgtttgacgtgccgcttcattatcagttccatgctgcatcgacacagggaggcggctatgatatgaggaaattgctgaacggtacggtcgtttccaagcatccgttgaaatcggttacatttgtcgataaccatgatacacagccggggcaatcgcttgagtcgactgtccaaacatggtttaagccgcttgcttacgcttttattctcacaagggaatctggataccctcaggttttctacggggatatgtacgggacgaaaggagactcccagcgcgaaattcctgccttgaaacacaaaattgaaccgatcttaaaagcgagaaaacagtatgcgtacggagcacagcatgattatttcgaccaccatgacattgtcggctggacaagggaaggcgacagctcggttgcaaattcaggtttggcggcattaataacagacggacccggtggggcaaagcgaatgtatgtcggccggcaaaacgccggtgagacatggcatgacattaccggaaaccgttcggagccggttgtcatcaattcggaaggctggggagagtttcacgtaaacggcgggtcggtttcaatttatgttcaaagatagacgcgtagggcccgcggctagcggccgcgtcgactagaagagcagagaggacggatttcctgaaggaaatccgtttttttattttgcccgtcttataaatttcgttgttcaataatcgcatccgattgcagtataaatttaacgatcactcatcatgttca

SEQ ID NO: 138 - DNA, 84 bp, synthetic construct
  source 1..84: mol_type = other DNA
atgatgaaaaaagtaagtggcttaatcatattatcgatgatgctgttgtctggtttttatatggaaacagcttatggtgcggct

SEQ ID NO: 139 - DNA, 87 bp, synthetic construct
  source 1..87: mol_type = other DNA
atgatgaaaaaagtaagtggcttaatcatattatcgatgatgctgttgtctggtttttatatggaaacagcttatggtgcggctgaa

SEQ ID NO: 140 - DNA, 90 bp, synthetic construct
  source 1..90: mol_type = other DNA
atgatgaaaaaagtaagtggcttaatcatattatcgatgatgctgttgtctggtttttatatggaaacagcttatggtgcggctgaagaa

SEQ ID NO: 141 - DNA, 93 bp, synthetic construct
  source 1..93: mol_type = other DNA
atgatgaaaaaagtaagtggcttaatcatattatcgatgatgctgttgtctggtttttatatggaaacagcttatggtgcggctgaagaagca

SEQ ID NO: 142 - DNA, 96 bp, synthetic construct
  source 1..96: mol_type = other DNA
atgatgaaaaaagtaagtggcttaatcatattatcgatgatgctgttgtctggtttttatatggaaacagcttatggtgcggctgaagaagcaaaa

SEQ ID NO: 143 - DNA, 99 bp, synthetic construct
  source 1..99: mol_type = other DNA
atgatgaaaaaagtaagtggcttaatcatattatcgatgatgctgttgtctggtttttatatggaaacagcttatggtgcggctgaagaagcaaaagaa

SEQ ID NO: 144 - DNA, 105 bp, synthetic construct
  source 1..105: mol_type = other DNA
atgatgaaaaaagtaagtggcttaatcatattatcgatgatgctgttgtctggtttttatatggaaacagcttatggtgcggctgaagaagcaaaagaaaaatat

SEQ ID NO: 145 - DNA, 108 bp, synthetic construct
  source 1..108: mol_type = other DNA
atgatgaaaaaagtaagtggcttaatcatattatcgatgatgctgttgtctggtttttatatggaaacagcttatggtgcggctgaagaagcaaaagaaaaatattta

SEQ ID NO: 146 - DNA, 111 bp, synthetic construct
  source 1..111: mol_type = other DNA
atgatgaaaaaagtaagtggcttaatcatattatcgatgatgctgttgtctggtttttatatggaaacagcttatggtgcggctgaagaagcaaaagaaaaatatttaatt

SEQ ID NO: 147 - DNA, 114 bp, synthetic construct
  source 1..114: mol_type = other DNA
atgatgaaaaaagtaagtggcttaatcatattatcgatgatgctgttgtctggtttttatatggaaacagcttatggtgcggctgaagaagcaaaagaaaaatatttaattggc

SEQ ID NO: 148 - DNA, 117 bp, synthetic construct
  source 1..117: mol_type = other DNA
atgatgaaaaaagtaagtggcttaatcatattatcgatgatgctgttgtctggtttttatatggaaacagcttatggtgcggctgaagaagcaaaagaaaaatatttaattggcttt

SEQ ID NO: 149 - DNA, 120 bp, synthetic construct
  source 1..120: mol_type = other DNA
atgatgaaaaaagtaagtggcttaatcatattatcgatgatgctgttgtctggtttttatatggaaacagcttatggtgcggctgaagaagcaaaagaaaaatatttaattggctttaat

SEQ ID NO: 150 - DNA, 123 bp, synthetic construct
  source 1..123: mol_type = other DNA
atgatgaaaaaagtaagtggcttaatcatattatcgatgatgctgttgtctggtttttatatggaaacagcttatggtgcggctgaagaagcaaaagaaaaatatttaattggctttaatgag

SEQ ID NO: 151 - DNA, 126 bp, synthetic construct
  source 1..126: mol_type = other DNA
atgatgaaaaaagtaagtggcttaatcatattatcgatgatgctgttgtctggtttttatatggaaacagcttatggtgcggctgaagaagcaaaagaaaaatatttaattggctttaatgagcag

SEQ ID NO: 152 - DNA, 102 bp, synthetic construct; identical to SEQ ID NO: 10
  source 1..102: mol_type = other DNA

SEQ ID NO: 153 - protein, 28 aa, synthetic construct
  SIGNAL 1..27
  REGION 28: note = SP-linker
MMKKVSGLIILSMMLLSGFYMETAYGAA

SEQ ID NO: 154 - protein, 29 aa, synthetic construct
  SIGNAL 1..27
  REGION 28..29: note = SP-linker
MMKKVSGLIILSMMLLSGFYMETAYGAAE

SEQ ID NO: 155 - protein, 30 aa, synthetic construct
  SIGNAL 1..27
  REGION 28..30: note = SP-linker
MMKKVSGLIILSMMLLSGFYMETAYGAAEE

SEQ ID NO: 156 - protein, 31 aa, synthetic construct
  SIGNAL 1..27
  REGION 28..31: note = SP-linker
MMKKVSGLIILSMMLLSGFYMETAYGAAEEA

SEQ ID NO: 157 - protein, 32 aa, synthetic construct
  SIGNAL 1..27
  REGION 28..32: note = SP-linker
MMKKVSGLIILSMMLLSGFYMETAYGAAEEAK

SEQ ID NO: 158 - protein, 33 aa, synthetic construct
  SIGNAL 1..27
  REGION 28..33: note = SP-linker
MMKKVSGLIILSMMLLSGFYMETAYGAAEEAKE

SEQ ID NO: 159 - protein, 35 aa, synthetic construct
  SIGNAL 1..27
  REGION 28..35: note = SP-linker
MMKKVSGLIILSMMLLSGFYMETAYGAAEEAKEKY

SEQ ID NO: 160 - protein, 36 aa, synthetic construct
  SIGNAL 1..27
  REGION 28..36: note = SP-linker
MMKKVSGLIILSMMLLSGFYMETAYGAAEEAKEKYL

SEQ ID NO: 161 - protein, 37 aa, synthetic construct
  SIGNAL 1..27
  REGION 28..37: note = SP-linker
MMKKVSGLIILSMMLLSGFYMETAYGAAEEAKEKYLI

SEQ ID NO: 162 - protein, 38 aa, synthetic construct
  SIGNAL 1..27
  REGION 28..38: note = SP-linker
MMKKVSGLIILSMMLLSGFYMETAYGAAEEAKEKYLIG

SEQ ID NO: 163 - protein, 39 aa, synthetic construct
  SIGNAL 1..27
  REGION 28..39: note = SP-linker
MMKKVSGLIILSMMLLSGFYMETAYGAAEEAKEKYLIGF

SEQ ID NO: 164 - protein, 40 aa, synthetic construct
  SIGNAL 1..27
  REGION 28..40: note = SP-linker
MMKKVSGLIILSMMLLSGFYMETAYGAAEEAKEKYLIGFN

SEQ ID NO: 165 - protein, 41 aa, synthetic construct
  SIGNAL 1..27
  REGION 28..41: note = SP-linker
MMKKVSGLIILSMMLLSGFYMETAYGAAEEAKEKYLIGFNE

SEQ ID NO: 166 - protein, 42 aa, synthetic construct
  SIGNAL 1..27
  REGION 28..42: note = SP-linker
MMKKVSGLIILSMMLLSGFYMETAYGAAEEAKEKYLIGFNEQ

SEQ ID NO: 167 - protein, 34 aa, synthetic construct; identical to SEQ ID NO: 12
  SIGNAL 1..27
  REGION 28..34: note = SP-linker

SEQ ID NO: 168 - DNA, 1539 bp, synthetic construct; identical to SEQ ID NO: 13
  source 1..1539: mol_type = other DNA

SEQ ID NO: 169 - DNA, 102 bp, synthetic construct
  source 1..102: mol_type = other DNA
atgatgaaaaaagtaagtggcttaatcatattatcgatgatgctgttgtctggtttttatatggaaacagcttatggtgcgacaggagcattaccgcagtct

SEQ ID NO: 170 - protein, 34 aa, synthetic construct
  SIGNAL 1..27
  REGION 28..34: note = SP-linker
MMKKVSGLIILSMMLLSGFYMETAYGATGALPQS

SEQ ID NO: 171 - protein, 31 aa, Aspergillus oryzae
MHLAIKSLFVSLLGASVLASPLPSNALVERA

SEQ ID NO: 172 - protein, 16 aa, Aspergillus oryzae
MKYSKLLLLLVSVVQA

SEQ ID NO: 173 - protein, 38 aa, synthetic construct
MHLAIKSLFVSLLGASVLASPLPSNALVERAFPAGNAT

SEQ ID NO: 174 - protein, 23 aa, synthetic construct
MKYSKLLLLLVSVVQAASGSGQS

SEQ ID NO: 175 - DNA, 21 bp, Thermomyces lanuginosus
  source 1..21: mol_type = genomic DNA
ttcccggcagggaatgccacg

SEQ ID NO: 176 - DNA, 21 bp, Thermothielavioides terrestris
  source 1..21: mol_type = genomic DNA
gccagtggcagtggccagtcc

SEQ ID NO: 177 - DNA, 93 bp, Aspergillus oryzae
  source 1..93: mol_type = genomic DNA
atgcatcttgctatcaagtctctctttgtctctctcctcggagccagcgttctcgcaagccctcttcccagcaatgctctggttgagagagcc

SEQ ID NO: 178 - DNA, 131 bp, Aspergillus oryzae
  source 1..131: mol_type = genomic DNA
atgaaggtacgtcaattccactgattaaacattatttgttacatacactccatcattgagtcaattataattaacacctcataattcagtactccaagcttctgctgctcctggtcagtgtggtccaggcc

SEQ ID NO: 179 - protein, 7 aa, Thermomyces lanuginosus
FPAGNAT

SEQ ID NO: 180 - protein, 7 aa, Thermothielavioides terrestris
ASGSGQS

SEQ ID NO: 181 - protein, 4 aa, Thermomyces lanuginosus
FPAG

SEQ ID NO: 182 - protein, 5 aa, Thermomyces lanuginosus
FPAGN

SEQ ID NO: 183 - protein, 6 aa, Thermomyces lanuginosus
FPAGNA

SEQ ID NO: 184 - protein, 4 aa, Thermothielavioides terrestris
ASGS

SEQ ID NO: 185 - protein, 5 aa, Thermothielavioides terrestris
ASGSG

SEQ ID NO: 186 - protein, 6 aa, Thermothielavioides terrestris
ASGSGQ

SEQ ID NO: 187 - DNA, 114 bp, synthetic construct
  source 1..114: mol_type = other DNA
atgcatcttgctatcaagtctctctttgtctctctcctcggagccagcgttctcgcaagccctcttcccagcaatgctctggttgagagagccttcccggcagggaatgccacg

SEQ ID NO: 188 - DNA, 152 bp, synthetic construct
  source 1..152: mol_type = other DNA
atgaaggtacgtcaattccactgattaaacattatttgttacatacactccatcattgagtcaattataattaacacctcataattcagtactccaagcttctgctgctcctggtcagtgtggtccaggccgccagtggcagtggccagtcc